European Patent Application EP 4 219 726 A1, published August 2, 2023. Title: SELF-COMPLEMNTARY ADENO-ASSOCIATED VIRUS VECTOR AND ITS USE IN TREATMENT OF MUSCULAR DYSTROPHY. Applicant: Research Institute at Nationwide Childrens Hospital. The sequence listing filed with the application follows.

SEQUENCE LISTING (15 sequences)

SEQ ID NO: 1 - DNA, 4511 bp, synthetic construct
  misc_feature 1..4511: note = scAAV construct sequence
  source 1..4511: mol_type = other DNA
ctgcgcgctcgctcgctcactgaggccgcccgggcaaagcccgggcgtcgggcgacctttggtcgcccggcctcagtgagcgagcgagcgcgcagagagggagtggccaactccatcactaggggttccttgtagttaatgattaacccgccatgctacttatctacgtagccatgctctagaggcgcgcccctgcaggacacacaaaaaaccaacacacagatctaatgaaaataaagatcttttattgcggccaagcttttaatgagtattcccacaagggttatcgctaatctgacatcccatattctggctggtgacctgcactttaaacagggtgccatcggcacacatgcacagcttatacctgacccaatctccggaccccagctggtctccactagaggagctgggcagtctggtagtggagaccatcacgctcccattcagaatgatgctgttttctgctttcagctccatgttgcctcccatgtgaaattcaattgtcttgcccatgatgaacacgccctcatttccccggacaatagctcgtccatccaccttgatattcaggtctgatgtagcgttactggtgattctctcagtgctggctttctggacgttcagagacttcaccccggaaggcagatgaaattcgtgtgtctcatagtcggtactgaacaggatattctgggtccggggatcaaagaactgcatgccaatgtcgctagtgattgatgttttattgttttccacagacagctttgtggttccctgctggaacacaatgggctgattgttcccggtgatcaccagattctcgtttctccgcccgccgacagtagatttgtacagtggatggatgacccccatatcggacacctgcttaaatcgcagcaggccactttcgtggaactccatagagtcacacccgtttgggccaatgcggatgacagcccaaatcaccagagtaatgatcagattaatcacggccaggataaacagcagaatgatgacgcagattgccaggtttcctttgcgccccctcaggcctgtcttatgcaggcgatcttcgtcaatagggatgtagccggctttgaaattgctgttgtgctccttattcactgatctcctctcgacggctttttctctcattgattttttcactggtccattgcttgactgctgctcggcggctgcggcggctgctgctgccatggtggtaccgggtacaattccgcagcttttagagcagaagtaacacttccgtacaggcctagaagtaaaggcaacatccactgaggagcagttctttgatttgcaccaccaccggatccgggacctgaaataaaagacaaaaagactaaacttacctgggcgcgccgctggctgctcctgagtgtctgtctgtgctgtggaggtggtggtagaatgagggcagcccctgtgcccctgggttatatagaggagcctacagggtgtgactagccaggaggggctgtccccagggaggggcccctgagagcagatgagctttcagctcgttgcccgggcaccgtgcccaccccggacccaggcgtgcagcttgcccagccccatggccttgtatgggctgccccaagggctgacttgctcactggttcctaaactaagtgctgagtctagctggcgggggacagctggcccttcgccgggaacatggaacagtaatactttgggagtcccaggcacgtataagccctggcccccaagcctgttacagcctgccctcagtcccccacagccttgttcgaagatcttcgcatgcaggggatccaccagggacagggttatttttagaggcagcaggtgttgggggggggggggcagccacatgtctgggttaattataaccaggcatctcgggtgtccccaggccttgcctccttacatgggcagcctagacccgtagtggggcatgctagacagcagggccccaaggtttgcccatgaaaggtctgttgccctcgcccctctggctccatggcctttttttagtccttgggcacattcctcctccccaaagggccgatgggcagatagaggagagacaggagcgtctcacaccacctcccctacccaggcccttacctcagttatttttaatctgaagggtctagcttagacatgcaagcttgcggccgccaattggttaaccccactccctctctgcgcgctcgctcgctcactgaggccgcccgggcaaagcccgggcgtcgggcgacctttggtcgcccggcctcagtgagcgagcgagcgcgcagagagggagtggggttaaccaattggcggccgcaagcttgcatgtctaagctagacccttcagattaaaaataactgaggtaagggcctgggtaggggaggtggtgtgagacgctcctgtctctcctctatctgcccatcggccctttggggaggaggaatgtgcccaaggactaaaaaaaggccatggagccagaggggcgagggcaacagacctttcatgggcaaaccttggggccctgctgtctagcatgccccactacgggtctaggctgcccatgtaaggaggcaaggcctggggacacccgagatgcctggttataattaacccagacatgtggctgcccccccccccccaacacctgctgcctctaaaaataaccctgtccctggtggatcccctgcatgcgaagatcttcgaacaaggctgtgggggactgagggcaggctgtaacaggcttgggggccagggcttatacgtgcctgggactcccaaagtattactgttccatgttcccggcgaagggccagctgtcccccgccagctagactcagcacttagtttaggaaccagtgagcaagtcagcccttggggcagcccatacaaggccatggggctgggcaagctgcacgcctgggtccggggtgggcacggtgcccgggcaacgagctgaaagctcatctgctctcaggggcccctccctggggacagcccctcctggctagtcacaccctgtaggctcctctatataacccaggggcacaggggctgccctcattctaccaccacctccacagcacagacagacactcaggagcagccagcggcgcgcccaggtaagtttagtctttttgtcttttatttcaggtcccggatccggtggtggtgcaaatcaaagaactgctcctcagtggatgttgcctttacttctaggcctgtacggaagtgttacttctgctctaaaagctgcggaattgtacccggtaccaccatggcagcagcagccgccgcagccgccgagcagcagtcaagcaatggaccagtgaaaaaatcaatgagagaaaaagccgtcgagaggagatcagtgaataaggagcacaacagcaatttcaaagccggctacatccctattgacgaagatcgcctgcataagacaggcctgagggggcgcaaaggaaacctggcaatctgcgtcatcattctgctgtttatcctggccgtgattaatctgatcattactctggtgatttgggctgtcatccgcattggcccaaacgggtgtgactctatggagttccacgaaagtggcctgctgcgatttaagcaggtgtccgatatgggggtcatccatccactgtacaaatctactgtcggcgggcggagaaacgagaatctggtgatcaccgggaacaatcagcccattgtgttccagcagggaaccacaaagctgtctgtggaaaacaataaaacatcaatcactagcgacattggcatgcagttctttgatccccggacccagaatatcctgttcagtaccgactatgagacacacgaatttcatctgccttccggggtgaagtctctgaacgtccagaaagccagcactgagagaatcaccagtaacgctacatcagacctgaatatcaaggtggatggacgagctattgtccggggaaatgagggcgtgttcatcatgggcaagacaattgaatttcacatgggaggcaacatggagctgaaagcagaaaacagcatcattctgaatgggagcgtgatggtctccactaccagactgcccagctcctctagtggagaccagctggggtccggagattgggtcaggtataagctgtgcatgtgtgccgatggcaccctgtttaaagtgcaggtcaccagccagaatatgggatgtcagattagcgataacccttgtgggaatactcattaaaagcttggccgcaataaaagatctttattttcattagatctgtgtgttggttttttgtgtgtcctgcaggggcgcgcctctagagcatggctacgtagataagtagcatggcgggttaatcattaactacaaggaacccctagtgatggagttggccactccctctctgcgcgctcgctcgctcactgaggccgggcgaccaaaggtcgcccgacgcccgggctttgcccgggcggcctcagtgagcgagcgagcgcgcag

SEQ ID NO: 2 - DNA, 957 bp, Homo sapiens
  source 1..957: mol_type = other DNA
atggcagcagcagccgccgcagccgccgagcagcagtcaagcaatggaccagtgaaaaaatcaatgagagaaaaagccgtcgagaggagatcagtgaataaggagcacaacagcaatttcaaagccggctacatccctattgacgaagatcgcctgcataagacaggcctgagggggcgcaaaggaaacctggcaatctgcgtcatcattctgctgtttatcctggccgtgattaatctgatcattactctggtgatttgggctgtcatccgcattggcccaaacgggtgtgactctatggagttccacgaaagtggcctgctgcgatttaagcaggtgtccgatatgggggtcatccatccactgtacaaatctactgtcggcgggcggagaaacgagaatctggtgatcaccgggaacaatcagcccattgtgttccagcagggaaccacaaagctgtctgtggaaaacaataaaacatcaatcactagcgacattggcatgcagttctttgatccccggacccagaatatcctgttcagtaccgactatgagacacacgaatttcatctgccttccggggtgaagtctctgaacgtccagaaagccagcactgagagaatcaccagtaacgctacatcagacctgaatatcaaggtggatggacgagctattgtccggggaaatgagggcgtgttcatcatgggcaagacaattgaatttcacatgggaggcaacatggagctgaaagcagaaaacagcatcattctgaatgggagcgtgatggtctccactaccagactgcccagctcctctagtggagaccagctggggtccggagattgggtcaggtataagctgtgcatgtgtgccgatggcaccctgtttaaagtgcaggtcaccagccagaatatgggatgtcagattagcgataacccttgtgggaatactcattaa

SEQ ID NO: 3 - protein, 318 aa, Homo sapiens
MAAAAAAAAEQQSSNGPVKKSMREKAVERRSVNKEHNSNFKAGYIPIDEDRLHKTGLRGRKGNLAICVIILLFILAVINLIITLVIWAVIRIGPNGCDSMEFHESGLLRFKQVSDMGVIHPLYKSTVGGRRNENLVITGNNQPIVFQQGTTKLSVENNKTSITSDIGMQFFDPRTQNILFSTDYETHEFHLPSGVKSLNVQKASTERITSNATSDLNIKVDGRAIVRGNEGVFIMGKTIEFHMGGNMELKAENSIILNGSVMVSTTRLPSSSSGDQLGSGDWVRYKLCMCADGTLFKVQVTSQNMGCQISDNPCGNTH

SEQ ID NO: 4 - DNA, 148 bp, synthetic construct
  misc_feature 1..148: note = 5' chimeric intron sequence
  source 1..148: mol_type = other DNA
gggtacaattccgcagcttttagagcagaagtaacacttccgtacaggcctagaagtaaaggcaacatccactgaggagcagttctttgatttgcaccaccaccggatccgggacctgaaataaaagacaaaaagactaaacttacct

SEQ ID NO: 5 - DNA, 792 bp, synthetic construct
  misc_feature 1..792: note = 5' MHCK7 promoter sequence
  source 1..792: mol_type = other DNA
gctggctgctcctgagtgtctgtctgtgctgtggaggtggtggtagaatgagggcagcccctgtgcccctgggttatatagaggagcctacagggtgtgactagccaggaggggctgtccccagggaggggcccctgagagcagatgagctttcagctcgttgcccgggcaccgtgcccaccccggacccaggcgtgcagcttgcccagccccatggccttgtatgggctgccccaagggctgacttgctcactggttcctaaactaagtgctgagtctagctggcgggggacagctggcccttcgccgggaacatggaacagtaatactttgggagtcccaggcacgtataagccctggcccccaagcctgttacagcctgccctcagtcccccacagccttgttcgaagatcttcgcatgcaggggatccaccagggacagggttatttttagaggcagcaggtgttgggggggggggggcagccacatgtctgggttaattataaccaggcatctcgggtgtccccaggccttgcctccttacatgggcagcctagacccgtagtggggcatgctagacagcagggccccaaggtttgcccatgaaaggtctgttgccctcgcccctctggctccatggcctttttttagtccttgggcacattcctcctccccaaagggccgatgggcagatagaggagagacaggagcgtctcacaccacctcccctacccaggcccttacctcagttatttttaatctgaagggtctagcttagacatgcaagctt

SEQ ID NO: 6 - DNA, 52 bp, synthetic construct
  misc_feature 1..52: note = 5' polyadenylation sequence
  source 1..52: mol_type = other DNA
acaaaaaaccaacacacagatctaatgaaaataaagatcttttattgcggcc

SEQ ID NO: 7 - DNA, 125 bp, synthetic construct
  misc_feature 1..125: note = 5' ITR
  source 1..125: mol_type = other DNA
aaccccactccctctctgcgcgctcgctcgctcactgaggccgcccgggcaaagcccgggcgtcgggcgacctttggtcgcccggcctcagtgagcgagcgagcgcgcagagagggagtggggtt

SEQ ID NO: 8 - DNA, 130 bp, synthetic construct
  misc_feature 1..130: note = 3' ITR 1
  source 1..130: mol_type = other DNA
ctgcgcgctcgctcgctcactgaggccgcccgggcaaagcccgggcgtcgggcgacctttggtcgcccggcctcagtgagcgagcgagcgcgcagagagggagtggccaactccatcactaggggttcct

SEQ ID NO: 9 - DNA, 720 bp, synthetic construct
  misc_feature 1..720: note = tMCK
  source 1..720: mol_type = other DNA
ccactacgggtctaggctgcccatgtaaggaggcaaggcctggggacacccgagatgcctggttataattaaccccaacacctgctgcccccccccccccaacacctgctgcctgagcctgagcggttaccccaccccggtgcctgggtcttaggctctgtacaccatggaggagaagctcgctctaaaaataaccctgtccctggtggatccactacgggtctaggctgcccatgtaaggaggcaaggcctggggacacccgagatgcctggttataattaaccccaacacctgctgcccccccccccccaacacctgctgcctgagcctgagcggttaccccaccccggtgcctgggtcttaggctctgtacaccatggaggagaagctcgctctaaaaataaccctgtccctggtggatccactacgggtctaggctgcccatgtaaggaggcaaggcctggggacacccgagatgcctggttataattaaccccaacacctgctgcccccccccccccaacacctgctgcctgagcctgagcggttaccccaccccggtgcctgggtcttaggctctgtacaccatggaggagaagctcgctctaaaaataaccctgtccctggtggatcctccctggggacagcccctcctggctagtcacaccctgtaggctcctctatataacccaggggcacaggggctgcccccgggtcac

SEQ ID NO: 10 - DNA, 43 bp, synthetic construct
  misc_feature 1..43: note = Hairpin
  source 1..43: mol_type = other DNA
cgcccgggcaaagcccgggcgtcgggcgacctttggtcgcccg

SEQ ID NO: 11 - DNA, 957 bp, synthetic construct
  misc_feature 1..957: note = 5' hSGCB DNA
  source 1..957: mol_type = other DNA
ttaatgagtattcccacaagggttatcgctaatctgacatcccatattctggctggtgacctgcactttaaacagggtgccatcggcacacatgcacagcttatacctgacccaatctccggaccccagctggtctccactagaggagctgggcagtctggtagtggagaccatcacgctcccattcagaatgatgctgttttctgctttcagctccatgttgcctcccatgtgaaattcaattgtcttgcccatgatgaacacgccctcatttccccggacaatagctcgtccatccaccttgatattcaggtctgatgtagcgttactggtgattctctcagtgctggctttctggacgttcagagacttcaccccggaaggcagatgaaattcgtgtgtctcatagtcggtactgaacaggatattctgggtccggggatcaaagaactgcatgccaatgtcgctagtgattgatgttttattgttttccacagacagctttgtggttccctgctggaacacaatgggctgattgttcccggtgatcaccagattctcgtttctccgcccgccgacagtagatttgtacagtggatggatgacccccatatcggacacctgcttaaatcgcagcaggccactttcgtggaactccatagagtcacacccgtttgggccaatgcggatgacagcccaaatcaccagagtaatgatcagattaatcacggccaggataaacagcagaatgatgacgcagattgccaggtttcctttgcgccccctcaggcctgtcttatgcaggcgatcttcgtcaatagggatgtagccggctttgaaattgctgttgtgctccttattcactgatctcctctcgacggctttttctctcattgattttttcactggtccattgcttgactgctgctcggcggctgcggcggctgctgctgccat

SEQ ID NO: 12 - DNA, 148 bp, synthetic construct
  misc_feature 1..148: note = 3' chimeric intron sequence Intron
  source 1..148: mol_type = other DNA
aggtaagtttagtctttttgtcttttatttcaggtcccggatccggtggtggtgcaaatcaaagaactgctcctcagtggatgttgcctttacttctaggcctgtacggaagtgttacttctgctctaaaagctgcggaattgtaccc

SEQ ID NO: 13 - DNA, 792 bp, synthetic construct
  misc_feature 1..792: note = 3' MHCK7 promoter sequence MHCK7
  source 1..792: mol_type = other DNA
aagcttgcatgtctaagctagacccttcagattaaaaataactgaggtaagggcctgggtaggggaggtggtgtgagacgctcctgtctctcctctatctgcccatcggccctttggggaggaggaatgtgcccaaggactaaaaaaaggccatggagccagaggggcgagggcaacagacctttcatgggcaaaccttggggccctgctgtctagcatgccccactacgggtctaggctgcccatgtaaggaggcaaggcctggggacacccgagatgcctggttataattaacccagacatgtggctgcccccccccccccaacacctgctgcctctaaaaataaccctgtccctggtggatcccctgcatgcgaagatcttcgaacaaggctgtgggggactgagggcaggctgtaacaggcttgggggccagggcttatacgtgcctgggactcccaaagtattactgttccatgttcccggcgaagggccagctgtcccccgccagctagactcagcacttagtttaggaaccagtgagcaagtcagcccttggggcagcccatacaaggccatggggctgggcaagctgcacgcctgggtccggggtgggcacggtgcccgggcaacgagctgaaagctcatctgctctcaggggcccctccctggggacagcccctcctggctagtcacaccctgtaggctcctctatataacccaggggcacaggggctgccctcattctaccaccacctccacagcacagacagacactcaggagcagccagc

SEQ ID NO: 14 - DNA, 54 bp, synthetic construct
  misc_feature 1..54: note = 3' polyadenylation sequence PolyA
  source 1..54: mol_type = other DNA
ggccgcaataaaagatctttattttcattagatctgtgtgttggttttttgtgt

SEQ ID NO: 15 - DNA, 130 bp, synthetic construct
  misc_feature 1..130: note = 3' ITR 2
  source 1..130: mol_type = other DNA
aggaacccctagtgatggagttggccactccctctctgcgcgctcgctcgctcactgaggccgggcgaccaaaggtcgcccgacgcccgggctttgcccgggcggcctcagtgagcgagcgagcgcgcag